European Patent Specification EP 3 129 067 B1, published January 4, 2023. Title: SITE-SPECIFIC GLYCOENGINEERING OF TARGETING MOIETIES. Applicant: GENZYME CORPORATION. The sequence listing filed with the application follows.

SEQUENCE LISTING (46 sequences)

SEQ ID NO: 1 - protein, 218 aa, Artificial Sequence
  source: /note="Description of Artificial Sequence: Synthetic polypeptide"
DIVMTQTPLSLSVTPGQPASISCKSSQSLLYSNGKTYLNWLLQKPGQSPQRLIYLVSKLDSGVPDRFSGSGSGTDFTLKISRVEAEDVGVYYCVQGTHLHTFGQGTRLEIKRTVAAPSVFIFPPSDEQLKSGTASVVCLLNNFYPREAKVQWKVDNALQSGNSQESVTEQDSKDSTYSLSSTLTLSKADYEKHKVYACEVTHQGLSSPVTKSFNRGEC

SEQ ID NO: 2 - protein, 443 aa, Artificial Sequence
  source: /note="Description of Artificial Sequence: Synthetic polypeptide"
VQLVESGGGLVQPGGSLRLSCAASGFTFNTYWMNWVRQAPGKGLEWVGQIRLKSNNYATHYAESVKGRFTISRDDSKNSLYLQMNSLKTEDTAVYYCTPVDFWGQGTTVTVSSASTKGPSVFPLAPSSKSTSGGTAALGCLVKDYFPEPVTVSWNSGALTSGVHTFPAVLQSSGLYSLSSVVTVPSSSLGTQTYICNVNHKPSNTKVDKKVEPKSCDKTHTCPPCPAPELLGGPSVFLFPPKPKDTLMISRTPEVTCVVVDVSHEDPEVKFNWYVDGVEVHNAKTKPREEQYNSTYRVVSVLTVLHQDWLNGKEYKCKVSNKALPAPIEKTISKAKGQPREPQVYTLPPSRDELTKNQVSLTCLVKGFYPSDIAVEWESNGQPENNYKTTPPVLDSDGSFFLYSKLTVDKSRWQQGNVFSCSVMHEALHNHYTQKSLSLSPGK

SEQ ID NO: 3 - protein, 444 aa, Artificial Sequence
  source: /note="Description of Artificial Sequence: Synthetic polypeptide"
EVQLVESGGGLVQPGGSLRLSCAASGFTFNTYWMNWVRQAPGKGLEWVGQIRLKSNNYATHYAESVKGRFTISRDDSKNSLYLQMNSLKTEDTAVYYCTPVDFWGQGTTVTVSSNSTKGPSVFPLAPSSKSTSGGTAALGCLVKDYFPEPVTVSWNSGALTSGVHTFPAVLQSSGLYSLSSVVTVPSSSLGTQTYICNVNHKPSNTKVDKKVEPKSCDKTHTCPPCPAPELLGGPSVFLFPPKPKDTLMISRTPEVTCVVVDVSHEDPEVKFNWYVDGVEVHNAKTKPREEQYNSTYRVVSVLTVLHQDWLNGKEYKCKVSNKALPAPIEKTISKAKGQPREPQVYTLPPSRDELTKNQVSLTCLVKGFYPSDIAVEWESNGQPENNYKTTPPVLDSDGSFFLYSKLTVDKSRWQQGNVFSCSVMHEALHNHYTQKSLSLSPGK

SEQ ID NO: 4 - protein, 444 aa, Artificial Sequence
  source: /note="Description of Artificial Sequence: Synthetic polypeptide"
EVQLVESGGGLVQPGGSLRLSCAASGFTFNTYWMNWVRQAPGKGLEWVGQIRLKSNNYATHYAESVKGRFTISRDDSKNSLYLQMNSLKTEDTAVYYCTPVDFWGQGTTVTVSSASTKGPSVFPLAPSSKSTSGGTAALGCLVKDYFPEPVTVSWNSGALTSGVHTFPAVLQSSGLYSLSSVVTVPSSSLGTQTYICNVNHKPSNTKVDKKVEPKSCDKTHTCPPCPAPELLGGPSVFLFPPKPKDTLMISRTPEVTCVVVDVSHEDPEVKFNWYVDGVEVHNAKTKPREEQYNSTYRVVSVLTVLHQDWLNGKEYKCKVSNKALPAPIEKTISKAKGQPREPQVYTLPPSRDELTKNQVSLTCLVKGFYPSDIAVEWESNGQPENNYKTTPPVLDSDGSFFLYSKLTVDKSRWQQGNVFSCSVMHEALHNHSTQKSLSLSPGK

SEQ ID NO: 5 - protein, 444 aa, Artificial Sequence
  source: /note="Description of Artificial Sequence: Synthetic polypeptide"
EVQLVESGGGLVQPGGSLRLSCAASGFTFNTYWMNWVRQAPGKGLEWVGQIRLKSNNYATHYAESVKGRFTISRDDSKNSLYLQMNSLKTEDTAVYYCTPVDFWGQGTTVTVSSASTKGPSVFPLAPSSKSTSGGTAALGCLVKDYFPEPVTVSWNSGALTSGVHTFPAVLQSSGLYSLSSVVTVPSSSLGTQTYICNVNHKPSNTKVDKKVEPKSCDKTHTCPPCPAPELLGGPSVFLFPPKPKDTLMISRTPEVTCVVVDVSHEDPEVKFNWYVDGVEVHNAKTKPREEQYNSTYRVVSVLTVLHQDWLNGKEYKCKVSNKALPAPIEKTISKAKGQPREPQVYTLPPSRDELTKNQVSLTCLVKGFYPSDIAVEWESNGQPENNYKTTPPVLDSDGSFFLYSKLTVDKSRWQQGNVFSCSVMHEALHNHYTQKNLSLSPGK

SEQ ID NO: 6 - protein, 444 aa, Artificial Sequence
  source: /note="Description of Artificial Sequence: Synthetic polypeptide"
EVQLVESGGGLVQPGGSLRLSCAASGFTFNTYWMNWVRQAPGKGLEWVGQIRLKSNNYATHYAESVKGRFTISRDDSKNSLYLQMNSLKTEDTAVYYCTPVDFWGQGTTVTVSSASTKGPSVFPLAPSSKSTSGGTAALGCLVKDYFPEPVTVSWNSGALTSGVHTFPAVLQSSGLYSLSSVVTVPSSSLGTQTYICNVNHKPSNTKVDKKVEPKSCDKTHTCPPCPAPELLGGPSVFLFPPKPKDTLMISRTPEVTCVVVDVSHEDPEVKFNWYVDGVEVHNAKTKPREEQYNSTYRVVSVLTVLHQDWLNGKEYKCKVSNKALPAPIEKTISKAKGQPREPQVYTLPPSRDELTKNQVSLTCLVKGFYPSDIAVEWESNGQPENNYKTTPPVLDSDGSFFLYSKLTVDKSRWQQGNVFSCSVMHEALHNHYTQKSLNLSPGK

SEQ ID NO: 7 - protein, 447 aa, Artificial Sequence
  source: /note="Description of Artificial Sequence: Synthetic polypeptide"
EVQLVESGGGLVQPGGSLRLSCAASGFTFNTYWMNWVRQAPGKGLEWVGQIRLKSNNYATHYAESVKGRFTISRDDSKNSLYLQMNSLKTEDTAVYYCTPVDFWGQGTTVTVSSASTKGPSVFPLAPSSKSTSGGTAALGCLVKDYFPEPVTVSWNSGALTSGVHTFPAVLQSSGLYSLSSVVTVPSSSLGTQTYICNVNHKPSNTKVDKKVEPKSCDKTHTCPPCPAPELLGGPSVFLFPPKPKDTLMISRTPEVTCVVVDVSHEDPEVKFNWYVDGVEVHNAKTKPREEQYNSTYRVVSVLTVLHQDWLNGKEYKCKVSNKALPAPIEKTISKAKGQPREPQVYTLPPSRDELTKNQVSLTCLVKGFYPSDIAVEWESNGQPENNYKTTPPVLDSDGSFFLYSKLTVDKSRWQQGNVFSCSVMHEALHNHYTQKSLSLSPGKNGT

SEQ ID NO: 8 - protein, 444 aa, Artificial Sequence
  source: /note="Description of Artificial Sequence: Synthetic polypeptide"
EVQLVESGGGLVQPGGSLRLSCAASGFTFNTYWMNWVRQAPGKGLEWVGQIRLKSNNYATHYAESVKGRFTISRDDSKNSLYLQMNSLKTEDTAVYYCTPVDFWGQGTTVTVSSASTKGPSVFPLAPSSKSTSGGTAALGCLVKDYFPEPVTVSWNSGALTSGVHTFPAVLQSSGLYSLSSVVTVPSSSLGTQTYICNVNHKPSNTKVDKKVEPKSCDKTHTCPPCPAPELLGGPSVFLFPPKPKDTLMISRTPEVTCVVVDVSHEDPEVKFNWYVDGVEVHNAKTKPREEQYNNTSRVVSVLTVLHQDWLNGKEYKCKVSNKALPAPIEKTISKAKGQPREPQVYTLPPSRDELTKNQVSLTCLVKGFYPSDIAVEWESNGQPENNYKTTPPVLDSDGSFFLYSKLTVDKSRWQQGNVFSCSVMHEALHNHYTQKSLSLSPGK

SEQ ID NO: 9 - protein, 215 aa, Artificial Sequence
  source: /note="Description of Artificial Sequence: Synthetic polypeptide"
EIVLTQSPGTLSLSPGERATLSCRASQSVSSSYLAWYQQKPGQAPRLLIYGASSRATGIPDRFSGSGSGTDFTLTISRLEPEDFAVYYCQQYGSSPWTFGQGTKVEIKRTVAAPSVFIFPPSDEQLKSGTASVVCLLNNFYPREAKVQWKVDNALQSGNSQESVTEQDSKDSTYSLSSTLTLSKADYEKHKVYACEVTHQGLSSPVTKSFNRGEC

SEQ ID NO: 10 - protein, 454 aa, Artificial Sequence
  source: /note="Description of Artificial Sequence: Synthetic polypeptide"
QVQLQESAPGLVKPSETLSLTCTVSGGSIRSYYWSWIRQPPGKGLEYIGYIYYTGSAIYNPSLQSRVTISVDTSKNQFSLKLNSVTAADTAVYYCAREGVRGASGYYYYGMDVWGQGTTVTVSSASTKGPSVFPLAPSSKSTSGGTAALGCLVKDYFPEPVTVSWNSGALTSGVHTFPAVLQSSGLYSLSSVVTVPSSSLGTQTYICNVNHKPSNTKVDKKVEPKSCDKTHTCPPCPAPELLGGPSVFLFPPKPKDTLMISRTPEVTCVVVDVSHEDPEVKFNWYVDGVEVHNAKTKPREEQYNSTYRVVSVLTVLHQDWLNGKEYKCKVSNKALPAPIEKTISKAKGQPREPQVYTLPPSRDELTKNQVSLTCLVKGFYPSDIAVEWESNGQPENNYKTTPPVLDSDGSFFLYSKLTVDKSRWQQGNVFSCSVMHEALHNHYTQKSLSLSPGK

SEQ ID NO: 11 - protein, 454 aa, Artificial Sequence
  source: /note="Description of Artificial Sequence: Synthetic polypeptide"
QVQLQESAPGLVKPSETLSLTCTVSGGSIRSYYWSWIRQPPGKGLEYIGYIYYTGSAIYNPSLQSRVTISVDTSKNQFSLKLNSVTAADTAVYYCAREGVRGASGYYYYGMDVWGQGTTVTVSSNSTKGPSVFPLAPSSKSTSGGTAALGCLVKDYFPEPVTVSWNSGALTSGVHTFPAVLQSSGLYSLSSVVTVPSSSLGTQTYICNVNHKPSNTKVDKKVEPKSCDKTHTCPPCPAPELLGGPSVFLFPPKPKDTLMISRTPEVTCVVVDVSHEDPEVKFNWYVDGVEVHNAKTKPREEQYNSTYRVVSVLTVLHQDWLNGKEYKCKVSNKALPAPIEKTISKAKGQPREPQVYTLPPSRDELTKNQVSLTCLVKGFYPSDIAVEWESNGQPENNYKTTPPVLDSDGSFFLYSKLTVDKSRWQQGNVFSCSVMHEALHNHYTQKSLSLSPGK

SEQ ID NO: 12 - protein, 214 aa, Artificial Sequence
  source: /note="Description of Artificial Sequence: Synthetic polypeptide"
DIQMTQSPSSLSASVGDRVTITCRASQDVNTAVAWYQQKPGKAPKLLIYSASFLYSGVPSRFSGSRSGTDFTLTISSLQPEDFATYYCQQHYTTPPTFGQGTKVEIKRTVAAPSVFIFPPSDEQLKSGTASVVCLLNNFYPREAKVQWKVDNALQSGNSQESVTEQDSKDSTYSLSSTLTLSKADYEKHKVYACEVTHQGLSSPVTKSFNRGEC

SEQ ID NO: 13 - protein, 450 aa, Artificial Sequence
  source: /note="Description of Artificial Sequence: Synthetic polypeptide"
EVQLVESGGGLVQPGGSLRLSCAASGFNIKDTYIHWVRQAPGKGLEWVARIYPTNGYTRYADSVKGRFTISADTSKNTAYLQMNSLRAEDTAVYYCSRWGGDGFYAMDYWGQGTLVTVSSASTKGPSVFPLAPSSKSTSGGTAALGCLVKDYFPEPVTVSWNSGALTSGVHTFPAVLQSSGLYSLSSVVTVPSSSLGTQTYICNVNHKPSNTKVDKKVEPKSCDKTHTCPPCPAPELLGGPSVFLFPPKPKDTLMISRTPEVTCVVVDVSHEDPEVKFNWYVDGVEVHNAKTKPREEQYNSTYRVVSVLTVLHQDWLNGKEYKCKVSNKALPAPIEKTISKAKGQPREPQVYTLPPSRDELTKNQVSLTCLVKGFYPSDIAVEWESNGQPENNYKTTPPVLDSDGSFFLYSKLTVDKSRWQQGNVFSCSVMHEALHNHYTQKSLSLSPGK

SEQ ID NO: 14 - protein, 450 aa, Artificial Sequence
  source: /note="Description of Artificial Sequence: Synthetic polypeptide"
EVQLVESGGGLVQPGGSLRLSCAASGFNIKDTYIHWVRQAPGKGLEWVARIYPTNGYTRYADSVKGRFTISADTSKNTAYLQMNSLRAEDTAVYYCSRWGGDGFYAMDYWGQGTLVTVSSNSTKGPSVFPLAPSSKSTSGGTAALGCLVKDYFPEPVTVSWNSGALTSGVHTFPAVLQSSGLYSLSSVVTVPSSSLGTQTYICNVNHKPSNTKVDKKVEPKSCDKTHTCPPCPAPELLGGPSVFLFPPKPKDTLMISRTPEVTCVVVDVSHEDPEVKFNWYVDGVEVHNAKTKPREEQYNSTYRVVSVLTVLHQDWLNGKEYKCKVSNKALPAPIEKTISKAKGQPREPQVYTLPPSRDELTKNQVSLTCLVKGFYPSDIAVEWESNGQPENNYKTTPPVLDSDGSFFLYSKLTVDKSRWQQGNVFSCSVMHEALHNHYTQKSLSLSPGK

SEQ ID NO: 15 - protein, 450 aa, Artificial Sequence
  source: /note="Description of Artificial Sequence: Synthetic polypeptide"
EVQLVESGGGLVQPGGSLRLSCAASGFNIKDTYIHWVRQAPGKGLEWVARIYPTNGYTRYADSVKGRFTISADTSKNTAYLQMNSLRAEDTAVYYCSRWGGDGFYAMDYWGQGTLVTVSSASTKGPSVFPLAPSSKSTSGGTAALGCLVKDYFPEPVTVSWNSGALTSGVHTFPAVLQSSGLYSLSSVVTVPSSSLGTQTYICNVNHKPSNTKVDKKVEPKSCDKTHTCPPCPAPELLGGPSVFLFPPKPKDTLMISRTPEVTCVVVDVSHEDPEVKFNWYVDGVEVHNAKTKPREEQYNNASRVVSVLTVLHQDWLNGKEYKCKVSNKALPAPIEKTISKAKGQPREPQVYTLPPSRDELTKNQVSLTCLVKGFYPSDIAVEWESNGQPENNYKTTPPVLDSDGSFFLYSKLTVDKSRWQQGNVFSCSVMHEALHNHYTQKSLSLSPGK

SEQ ID NO: 16 - protein, 450 aa, Artificial Sequence
  source: /note="Description of Artificial Sequence: Synthetic polypeptide"
EVQLVESGGGLVQPGGSLRLSCAASGFNIKDTYIHWVRQAPGKGLEWVARIYPTNGYTRYADSVKGRFTISADTSKNTAYLQMNSLRAEDTAVYYCSRWGGDGFYAMDYWGQGTLVTVSSNSTKGPSVFPLAPSSKSTSGGTAALGCLVKDYFPEPVTVSWNSGALTSGVHTFPAVLQSSGLYSLSSVVTVPSSSLGTQTYICNVNHKPSNTKVDKKVEPKSCDKTHTCPPCPAPELLGGPSVFLFPPKPKDTLMISRTPEVTCVVVDVSHEDPEVKFNWYVDGVEVHNAKTKPREEQYNNASRVVSVLTVLHQDWLNGKEYKCKVSNKALPAPIEKTISKAKGQPREPQVYTLPPSRDELTKNQVSLTCLVKGFYPSDIAVEWESNGQPENNYKTTPPVLDSDGSFFLYSKLTVDKSRWQQGNVFSCSVMHEALHNHYTQKSLSLSPGK

SEQ ID NO: 17-22 - skipped (6 entries)

SEQ ID NO: 23 - protein, 213 aa, Artificial Sequence
  source: /note="Description of Artificial Sequence: Synthetic polypeptide"
EIVLTQSPATLSLSPGERATLSCSATSSVSYMHWYQQKPGQAPRRLIYDTSKLASGVPARFSGSGSGTSYTLTISSLEPEDFAVYYCQQWSSNPLTFGGGTKVEIKRTVAAPSVFIFPPSDEQLKSGTASVVCLLNNFYPREAKVQWKVDNALQSGNSQESVTEQDSKDSTYSLSSTLTLSKADYEKHKVYACEVTHQGLSSPVTKSFNRGEC

SEQ ID NO: 24 - protein, 450 aa, Artificial Sequence
  source: /note="Description of Artificial Sequence: Synthetic polypeptide"
EVQLLQSGGGLVQPGGSLRLSCAASGYKFTSYVMHWVRQAPGKGLEWVGYINPYNDVTKYNEKFKGRFTLSRDNSKNTLYLQMNSLRAEDTAVYYCARGSYYDYDGFVYWGQGTLVTVSSASTKGPSVFPLAPSSKSTSGGTAALGCLVKDYFPEPVTVSWNSGALTSGVHTFPAVLQSSGLYSLSSVVTVPSSSLGTQTYICNVNHKPSNTKVDKKVEPKSCDKTHTCPPCPAPELLGGPSVFLFPPKPKDTLMISRTPEVTCVVVDVSHEDPEVKFNWYVDGVEVHNAKTKPREEQYNSTYRVVSVLTVLHQDWLNGKEYKCKVSNKALPAPIEKTISKAKGQPREPQVYTLPPSRDELTKNQVSLTCLVKGFYPSDIAVEWESNGQPENNYKTTPPVLDSDGSFFLYSKLTVDKSRWQQGNVFSCSVMHEALHNHYTQKSLSLSPGK

SEQ ID NO: 25 - protein, 450 aa, Artificial Sequence
  source: /note="Description of Artificial Sequence: Synthetic polypeptide"
EVQLLQSGGGLVQPGGSLRLSCAASGYKFTSYVMHWVRQAPGKGLEWVGYINPYNDVTKYNEKFKGRFTLSRDNSKNTLYLQMNSLRAEDTAVYYCARGSYYDYDGFVYWGQGTLVTVSSASTKGPSVFPLAPSSKSTSGGTAALGCLVKDYFPEPVTVSWNSGALTSGVHTFPAVLQSSGLYSLSSVVTVPSSSLGTQTYICNVNHKPSNTKVDKKVEPKSCDKTHTCPPCPAPELLGGPSVFLFPPKPKDTLMISRTPEVTCVVVDVSHEDPEVKFNWYVDGVEVHNAKTKPREEQYNNTSRVVSVLTVLHQDWLNGKEYKCKVSNKALPAPIEKTISKAKGQPREPQVYTLPPSRDELTKNQVSLTCLVKGFYPSDIAVEWESNGQPENNYKTTPPVLDSDGSFFLYSKLTVDKSRWQQGNVFSCSVMHEALHNHYTQKSLSLSPGK

SEQ ID NO: 26 - protein, 450 aa, Artificial Sequence
  source: /note="Description of Artificial Sequence: Synthetic polypeptide"
EVQLLQSGGGLVQPGGSLRLSCAASGYKFTSYVMHWVRQAPGKGLEWVGYINPYNDVTKYNEKFKGRFTLSRDNSKNTLYLQMNSLRAEDTAVYYCARGSYYDYDGFVYWGQGTLVTVSSASTKGPSVFPLAPSSKSTSGGTAALGCLVKDYFPEPVTVSWNSGALTSGVHTFPAVLQSSGLYSLSSVVTVPSSSLGTQTYICNVNHKPSNTKVDKKVEPKSCDKTHTCPPCPAPELLGGPSVFLFPPKPKDTLMISRTPEVTCVVVDVSHEDPEVKFNWYVDGVEVHNAKTKPREEQYNNASRVVSVLTVLHQDWLNGKEYKCKVSNKALPAPIEKTISKAKGQPREPQVYTLPPSRDELTKNQVSLTCLVKGFYPSDIAVEWESNGQPENNYKTTPPVLDSDGSFFLYSKLTVDKSRWQQGNVFSCSVMHEALHNHYTQKSLSLSPGK

SEQ ID NO: 27 - protein, 450 aa, Artificial Sequence
  source: /note="Description of Artificial Sequence: Synthetic polypeptide"
EVQLLQSGGGLVQPGGSLRLSCAASGYKFTSYVMHWVRQAPGKGLEWVGYINPYNDVTKYNEKFKGRFTLSRDNSKNTLYLQMNSLRAEDTAVYYCARGSYYDYDGFVYWGQGTLVTVSSASTKGPSVFPLAPSSKSTSGGTAALGCLVKDYFPEPVTVSWNSGALTSGVHTFPAVLQSSGLYSLSSVVTVPSSSLGTQTYICNVNHKPSNTKVDKKVEPKSCDKTHTCPPCPAPELLGGPSVFLFPPKPKDTLMISRTPEVTCVVVDVSHEDPEVKFNWYVDGVEVHNAKTKPREEQYQNTSRVVSVLTVLHQDWLNGKEYKCKVSNKALPAPIEKTISKAKGQPREPQVYTLPPSRDELTKNQVSLTCLVKGFYPSDIAVEWESNGQPENNYKTTPPVLDSDGSFFLYSKLTVDKSRWQQGNVFSCSVMHEALHNHYTQKSLSLSPGK

SEQ ID NO: 28 - protein, 218 aa, Artificial Sequence; identical to SEQ ID NO: 1
  source: /note="Description of Artificial Sequence: Synthetic polypeptide"

SEQ ID NO: 29 - protein, 444 aa, Artificial Sequence
  source: /note="Description of Artificial Sequence: Synthetic polypeptide"
EVQLVESGGGLVQPGGSLRLSCAASGFTFNTYWMNWVRQAPGKGLEWVGQIRLKSNNYATHYAESVKGRFTISRDDSKNSLYLQMNSLKTEDTAVYYCTPVDFWGQGTTVTVSSASTKGPSVFPLAPSSKSTSGGTAALGCLVKDYFPEPVTVSWNSGALTSGVHTFPAVLQSSGLYSLSSVVTVPSSSLGTQTYICNVNHKPSNTKVDKKVEPKSCDKTHTCPPCPAPELLGGPSVFLFPPKPKDTLMISRTPEVTCVVVDVSHEDPEVKFNWYVDGVEVHNAKTKPREEQYNSTYRVVSVLTVLHQDWLNGKEYKCKVSNKALPAPIEKTISKAKGQPREPQVYTLPPSRDELTKNQVSLTCLVKGFYPSDIAVEWESNGQPENNYKTTPPVLDSDGSFFLYSKLTVDKSRWQQGNVFSCSVMHEALHNHYTQKSLSLSPGK

SEQ ID NO: 30 - protein, 444 aa, Artificial Sequence; identical to SEQ ID NO: 8
  source: /note="Description of Artificial Sequence: Synthetic polypeptide"

SEQ ID NO: 31 - protein, 218 aa, Artificial Sequence
  source: /note="Description of Artificial Sequence: Synthetic polypeptide"
DIVMTQTPLSLSVTPGQPASISCKSSQSLLYSNGKTYLNWVLQKPGQSPQRLIYLVSKLDSGVPDRFSGSGSGTDFTLKISRVEAEDVGVYYCVQGSHFHTFGQGTKLEIKRTVAAPSVFIFPPSDEQLKSGTASVVCLLNNFYPREAKVQWKVDNALQSGNSQESVTEQDSKDSTYSLSSTLTLSKADYEKHKVYACEVTHQGLSSPVTKSFNRGEC

SEQ ID NO: 32 - protein, 444 aa, Artificial Sequence
  source: /note="Description of Artificial Sequence: Synthetic polypeptide"
EVQLVESGGGLVQPGGSLRLSCAASGFPFSNYWMNWVRQAPGKGLEWVGQIRLKSNNYATHYAESVKGRFTISRDDSKNSLYLQMNSLKTEDTAVYYCTPIDYWGQGTTVTVSSASTKGPSVFPLAPSSKSTSGGTAALGCLVKDYFPEPVTVSWNSGALTSGVHTFPAVLQSSGLYSLSSVVTVPSSSLGTQTYICNVNHKPSNTKVDKKVEPKSCDKTHTCPPCPAPELLGGPSVFLFPPKPKDTLMISRTPEVTCVVVDVSHEDPEVKFNWYVDGVEVHNAKTKPREEQYNSTYRVVSVLTVLHQDWLNGKEYKCKVSNKALPAPIEKTISKAKGQPREPQVYTLPPSRDELTKNQVSLTCLVKGFYPSDIAVEWESNGQPENNYKTTPPVLDSDGSFFLYSKLTVDKSRWQQGNVFSCSVMHEALHNHYTQKSLSLSPGK

SEQ ID NO: 33 - protein, 444 aa, Artificial Sequence
  source: /note="Description of Artificial Sequence: Synthetic polypeptide"
EVQLVESGGGLVQPGGSLRLSCAASGFPFSNYWMNWVRQAPGKGLEWVGQIRLKSNNYATHYAESVKGRFTISRDDSKNSLYLQMNSLKTEDTAVYYCTPIDYWGQGTTVTVSSASTKGPSVFPLAPSSKSTSGGTAALGCLVKDYFPEPVTVSWNSGALTSGVHTFPAVLQSSGLYSLSSVVTVPSSSLGTQTYICNVNHKPSNTKVDKKVEPKSCDKTHTCPPCPAPELLGGPSVFLFPPKPKDTLMISRTPEVTCVVVDVSHEDPEVKFNWYVDGVEVHNAKTKPREEQYNNTSRVVSVLTVLHQDWLNGKEYKCKVSNKALPAPIEKTISKAKGQPREPQVYTLPPSRDELTKNQVSLTCLVKGFYPSDIAVEWESNGQPENNYKTTPPVLDSDGSFFLYSKLTVDKSRWQQGNVFSCSVMHEALHNHYTQKSLSLSPGK

SEQ ID NO: 34 - protein, 444 aa, Artificial Sequence
  source: /note="Description of Artificial Sequence: Synthetic polypeptide"
EVQLVESGGGLVQPGGSLRLSCAASGFPFSNYWMNWVRQAPGKGLEWVGQIRLKSNNYATHYAESVKGRFTISRDDSKNSLYLQMNSLKTEDTAVYYCTPIDYWGQGTTVTVSSASTKGPSVFPLAPSSKSTSGGTAALGCLVKDYFPEPVTVSWNSGALTSGVHTFPAVLQSSGLYSLSSVVTVPSSSLGTQTYICNVNHKPSNTKVDKKVEPKSCDKTHTCPPCPAPELLGGPSVFLFPPKPKDTLMISRTPEVTCVVVDVSHEDPEVKFNWYVDGVEVHNAKTKPREEQYNNASRVVSVLTVLHQDWLNGKEYKCKVSNKALPAPIEKTISKAKGQPREPQVYTLPPSRDELTKNQVSLTCLVKGFYPSDIAVEWESNGQPENNYKTTPPVLDSDGSFFLYSKLTVDKSRWQQGNVFSCSVMHEALHNHYTQKSLSLSPGK

SEQ ID NO: 35 - protein, 444 aa, Artificial Sequence
  source: /note="Description of Artificial Sequence: Synthetic polypeptide"
EVQLVESGGGLVQPGGSLRLSCAASGFPFSNYWMNWVRQAPGKGLEWVGQIRLKSNNYATHYAESVKGRFTISRDDSKNSLYLQMNSLKTEDTAVYYCTPIDYWGQGTTVTVSSASTKGPSVFPLAPSSKSTSGGTAALGCLVKDYFPEPVTVSWNSGALTSGVHTFPAVLQSSGLYSLSSVVTVPSSSLGTQTYICNVNHKPSNTKVDKKVEPKSCDKTHTCPPCPAPELLGGPSVFLFPPKPKDTLMISRTPEVTCVVVDVSHEDPEVKFNWYVDGVEVHNAKTKPREEQYQNTSRVVSVLTVLHQDWLNGKEYKCKVSNKALPAPIEKTISKAKGQPREPQVYTLPPSRDELTKNQVSLTCLVKGFYPSDIAVEWESNGQPENNYKTTPPVLDSDGSFFLYSKLTVDKSRWQQGNVFSCSVMHEALHNHYTQKSLSLSPGK

SEQ ID NO: 36 - protein, 214 aa, Artificial Sequence; identical to SEQ ID NO: 12
  source: /note="Description of Artificial Sequence: Synthetic polypeptide"

SEQ ID NO: 37 - protein, 450 aa, Artificial Sequence; identical to SEQ ID NO: 13
  source: /note="Description of Artificial Sequence: Synthetic polypeptide"

SEQ ID NO: 38 - protein, 450 aa, Artificial Sequence; identical to SEQ ID NO: 15
  source: /note="Description of Artificial Sequence: Synthetic polypeptide"

SEQ ID NO: 39 - protein, 4 aa, Artificial Sequence
  source: /note="Description of Artificial Sequence: Synthetic peptide"
NNAS

SEQ ID NO: 40 - protein, 4 aa, Artificial Sequence
  source: /note="Description of Artificial Sequence: Synthetic peptide"
GGGG

SEQ ID NO: 41 - protein, 5 aa, Artificial Sequence
  source: /note="Description of Artificial Sequence: Synthetic peptide"
GGGGG

SEQ ID NO: 42 - protein, 6 aa, Artificial Sequence
  source: /note="Description of Artificial Sequence: Synthetic peptide"
GGGGGG

SEQ ID NO: 43 - protein, 7 aa, Artificial Sequence
  source: /note="Description of Artificial Sequence: Synthetic peptide"
GGGGGGG

SEQ ID NO: 44 - protein, 8 aa, Artificial Sequence
  source: /note="Description of Artificial Sequence: Synthetic peptide"
GGGGGGGG

SEQ ID NO: 45 - protein, 5 aa, Artificial Sequence
  source: /note="Description of Artificial Sequence: Synthetic peptide"
GGGGS

SEQ ID NO: 46 - protein, 10 aa, Artificial Sequence
  source: /note="Description of Artificial Sequence: Synthetic peptide"
GGGGSGGGGS